European Patent Application EP 4 316 525 A1, published February 7, 2024. Title: CONJUGATE, PREPARATION METHOD THEREOF AND USE THEREOF. Applicant: NANKAI UNIVERSITY. The sequence listing filed with the application follows.

SEQUENCE LISTING (5 sequences)

SEQ ID NO: 1 - RNA, 21 nt, Artificial sequence
cauguuguucagcugcugcuu

SEQ ID NO: 2 - RNA, 21 nt, Artificial sequence
cauguuguucagcugcugcuu

SEQ ID NO: 3 - RNA, 21 nt, Artificial sequence
gcagcagcugaacaacauguu

SEQ ID NO: 4 - RNA, 21 nt, Artificial sequence
gcgacgaccuuacagagcguu

SEQ ID NO: 5 - RNA, 21 nt, Artificial sequence
cgcucuguaaggucgucgcuu